European Patent Specification EP 3 924 512 B1, published July 12, 2023. Title: PROTOCOLS AND KITS FOR MULTIPLEX AMPLIFICATION AND NGS-SPECIFIC TAGGING. Applicant: Biocartis NV. The sequence listing filed with the application follows.

SEQUENCE LISTING (8 sequences)

SEQ ID NO: 1 - DNA, 22 bp, Artificial Sequence
  Anisotropical hairpin primer forward
acgggcggcctgcgctgtccga

SEQ ID NO: 2 - DNA, 23 bp, Artificial Sequence
  Anisotropical hairpin primer reverse
agcgtggggtgtcgcctcgcgca

SEQ ID NO: 3 - DNA, 21 bp, Artificial Sequence
  Isotropical hairpin primer forward
tcggtcggcctccgcgaccga

SEQ ID NO: 4 - DNA, 21 bp, Artificial Sequence
  Isotropical hairpin primer reverse
cgcgcgactgtgcctcgcgca

SEQ ID NO: 5 - DNA, 132 bp, Artificial Sequence
  Anisotropical appended amplicon from BRAF H.sapiens sequence
acgggcggcctgcgctgtccgatgggcagattacagagggacaagaattggatctggatcatttggaacagtctacaagggaaagtggcatggtaagtatgtaatgtggtgcgcgaggcgacaccccacgct

SEQ ID NO: 6 - DNA, 139 bp, Artificial Sequence
  Anisotropical appended amplicon from KRAS H.sapiens sequence
acgggcggcctgcgctgtccgatgatggagaaacctgtctcttggatattctcgacacagcaggtcaagaggagtacagtgcaatgagggaccagtacatgaggactggggagggctgcgcgaggcgacaccccacgct

SEQ ID NO: 7 - DNA, 143 bp, Artificial Sequence
  Anisotropical appended amplicon from ERBB2 H.sapiens sequence
acgggcggcctgcgctgtccgatgtggctacatgttcctgatctccttagacaactacctttctacggacgtgggatcctgcaccctcgtctgccccctgcacaaccaagaggtgacagctgcgcgaggcgacaccccacgct

SEQ ID NO: 8 - DNA, 143 bp, Artificial Sequence
  Anisotropical appended amplicon from ERBB2 H.sapiens sequence
acgggcggcctgcgctgtccgaccataccctctcagcgtacccttgtccccaggaagcatacgtgatggctggtgtgggctccccatatgtctcccgcctttctgggcatctgcctgacatgcgcgaggcgacaccccacgct